European Patent Application EP 4 242 312 A1, published September 13, 2023. Title: Microorganisms with increased production capacity of 3-hydroxypropionic acid from glucose orand uses thereof. Applicant: LG CHEM, LTD. The sequence listing filed with the application follows.

SEQUENCE LISTING (25 sequences)

SEQ ID NO: 1 - DNA, 57 bp, Artificial Sequence
  GPD1-F
catcatcatggatccatagcagtaagaaaggagcatccatcatgagcgctgcggctg

SEQ ID NO: 2 - DNA, 49 bp, Artificial Sequence
  GPD1-R
catcatcatgagctctcaatcttcatgaaggtctaattcttcaatcatg

SEQ ID NO: 3 - DNA, 62 bp, Artificial Sequence
  GPP2-F
catcatcatggtaccacagttttagtaaaggagcatcaaaaatgggactcactacgaaaccg

SEQ ID NO: 4 - DNA, 41 bp, Artificial Sequence
  GPP2-R
catcatcatctcgagttaccatttcagcagatcgtctttgg

SEQ ID NO: 5 - DNA, 114 bp, Artificial Sequence
  LTTR
gtcagcctcagcgcacctcgaatgtgcaaaaacgcagaccatacttgcacatcaccgcattgagtacatcaaaaatgcactgttaggatcgatccagacaacaaaaaagccaca

SEQ ID NO: 6 - DNA, 35 bp, Artificial Sequence
  dhaB-gdrA-F
gaattcatgaaaagatcaaaacgatttgcagtcct

SEQ ID NO: 7 - DNA, 29 bp, Artificial Sequence
  dhaB-gdrA-R
aagcttgatctcccactgaccaaagctgg

SEQ ID NO: 8 - DNA, 38 bp, Artificial Sequence
  gdrB-F
aagcttagagggggccgtcatgtcgctttcaccgccag

SEQ ID NO: 9 - DNA, 28 bp, Artificial Sequence
  gdrB-R
cttaagtcagtttctctcacttaacggc

SEQ ID NO: 10 - DNA, 26 bp, Artificial Sequence
  aldH-F
ggtaccatgaattttcatcatctggc

SEQ ID NO: 11 - DNA, 24 bp, Artificial Sequence
  aldH-R
catatgtcaggcctccaggcttat

SEQ ID NO: 12 - DNA, 39 bp, Artificial Sequence
  btuR-F
tggaggcctgacataatgagtgatgaacgctaccaacag

SEQ ID NO: 13 - DNA, 39 bp, Artificial Sequence
  btuR-R
ttgagatctgccatattaataatcgatccctatctgcgc

SEQ ID NO: 14 - DNA, 20 bp, Artificial Sequence
  ptsG-1000-F
acgcgatgtgaaattttgtc

SEQ ID NO: 15 - DNA, 53 bp, Artificial Sequence
  ptsG-1000-R
cactatacctaggactgagctagccgtaaaaattgagagtgctcctgagtatg

SEQ ID NO: 16 - DNA, 19 bp, Artificial Sequence
  J23-over-F
tttacggctagctcagtcc

SEQ ID NO: 17 - DNA, 24 bp, Artificial Sequence
  glk-over-R
ttacagaatgtgacctaaggtctg

SEQ ID NO: 18 - DNA, 52 bp, Artificial Sequence
  ptsG+1000-F
catttacgccagaccttaggtcacattctgtaatccgtaagacgttggggag

SEQ ID NO: 19 - DNA, 18 bp, Artificial Sequence
  ptsG+1000-R
ccaacatcttcccggatg

SEQ ID NO: 20 - DNA, 40 bp, Artificial Sequence
  galP_infu_F
tagtgctagcggtacatgcctgacgctaaaaaacaggggc

SEQ ID NO: 21 - DNA, 31 bp, Artificial Sequence
  galP_infu_R
gtcaaaataattaatcgtgagcgcctatttc

SEQ ID NO: 22 - DNA, 33 bp, Artificial Sequence
  glk_infu_F
tcacgattaattattttgactttagcggagcag

SEQ ID NO: 23 - DNA, 45 bp, Artificial Sequence
  glk_infu_R
tccaattgagatctgccatattacagaatgtgacctaaggtctgg

SEQ ID NO: 24 - DNA, 32 bp, Artificial Sequence
  TAC
ttgacaattaatcatcggctcgtataatgtgt

SEQ ID NO: 25 - DNA, 166 bp, Artificial Sequence
  BAD
aaagccatgacaaaaacgcgtaacaaaagtgtctataatcacggcagaaaagtccacattgattatttgcacggcgtcacactttgctatgccatagcatttttatccataagattagcggatcctacctgacgctttttatcgcaactctctactgtttctccat